European Patent Application EP 4 607 196 A2, published August 27, 2025. Title: INSILICO METHOD AND SYSTEM FOR DESIGNING A BASELINE PEPTIDE BIORECEPTOR FOR SENSING A BIOMARKER FOR DYSGLYCEMIC DISORDER. Applicant: Tata Consultancy Services Limited. Application IN 202421013153, filed February 23, 2023. The sequence listing filed with the application follows.

SEQUENCE LISTING (1 sequence)

SEQ ID NO: 1 - protein, 36 aa, synthetic construct
CQLIQMDYVGBGTAFFILPBZGMBTVIALSRDTIDR